European Patent Application EP 4 501 950 A1, published February 5, 2025. Title: HIGH-AFFINITY TCR FOR IDENTIFYING MAGE-A4 ANTIGEN, AND SEQUENCE AND USE THEREOF. Applicant: XLIFESC, LTD. Application EP 23774013.9, filed March 24, 2023. The sequence listing filed with the application follows.

SEQUENCE LISTING (62 sequences)

SEQ ID NO: 1 - protein, 111 aa, synthetic construct
GEDVEQSLFLSVREGDSSVINCTYTDSSSTYLYWYKQEPGAGLQLLTYIFSNMDMKQDQRLTVLLNKKDKHLSLRIADTQTGDSAIYFCAEQSFGNEKLTFGTGTRLTIIP

SEQ ID NO: 2 - protein, 112 aa, synthetic construct
NAGVTQTPKFRVLKTGQSMTLLCAQDMNHEYMYWYRQDPGMGLRLIHYSVGEGTTAKGEVPDGYNVSRLKKQNFLLGLESAAPSQTSVYFCASSLGRAYEQYFGPGTRLTVT

SEQ ID NO: 3 - protein, 111 aa, synthetic construct
GEDVEQSLSLSVREGDSVVINCTYTDSSSTYLYWYKQEPGAGLQLLTYIFSNMDMKQDQRLTVLLNKKDKHLSLRIADVQTGDSAIYFCAEQSFGNEKLTFGTGTRLTVTP

SEQ ID NO: 4 - protein, 112 aa, synthetic construct
NAGVTQTPKYLSVKTGQSVTLLCAQDMNHEYMYWYRQDPGQGLRLIHYSVGEGTTAKGEVPDRYNVSRLKKQNFLLGIESVTPSDTSVYFCASSLGRAYEQYFGPGTRLTVT

SEQ ID NO: 5 - DNA, 333 bp, synthetic construct
  source 1..333: mol_type = other DNA
ggtgaagatgttgaacaaagcctgagcctgagcgtgcgcgaaggcgatagcgtggttattaattgcacctataccgatagtagcagtacctatctgtattggtataaacaggaaccgggcgcaggtctgcagctgctgacctatattttcagtaatatggatatgaagcaggatcagcgcctgaccgttctgctgaataagaaagataaacatctgagcctgcgtattgccgatgttcagaccggtgacagcgcaatctatttctgtgccgaacagagttttggcaatgaaaagctgacctttggtaccggtacccgtctgaccgttaccccg

SEQ ID NO: 6 - DNA, 336 bp, synthetic construct
  source 1..336: mol_type = other DNA
aatgccggtgttacccagaccccgaaatatctgagcgttaaaaccggccagagtgttaccctgctgtgcgcccaggatatgaatcatgaatatatgtattggtaccgccaggaccctggccagggtctgcgcttaattcattatagtgtgggtgaaggtaccaccgcaaaaggcgaagtgccggatcgttataatgtgagtcgcctgaagaaacagaattttctgctgggcattgaaagtgtgaccccgagtgataccagcgtgtatttctgtgcaagtagcctgggtcgtgcctatgaacagtattttggcccgggtacccgcctgaccgtgacc

SEQ ID NO: 7 - protein, 24 aa, synthetic construct
GGGSEGGGSEGGGSEGGGSEGGTG

SEQ ID NO: 8 - DNA, 72 bp, synthetic construct
  source 1..72: mol_type = other DNA
ggtggcggcagtgaaggcggtggtagcgaaggcggcggcagcgaaggtggtggtagtgaaggtggtaccggc

SEQ ID NO: 9 - protein, 247 aa, synthetic construct
GEDVEQSLSLSVREGDSVVINCTYTDSSSTYLYWYKQEPGAGLQLLTYIFSNMDMKQDQRLTVLLNKKDKHLSLRIADVQTGDSAIYFCAEQSFGNEKLTFGTGTRLTVTPGGGSEGGGSEGGGSEGGGSEGGTGNAGVTQTPKYLSVKTGQSVTLLCAQDMNHEYMYWYRQDPGQGLRLIHYSVGEGTTAKGEVPDRYNVSRLKKQNFLLGIESVTPSDTSVYFCASSLGRAYEQYFGPGTRLTVT

SEQ ID NO: 10 - DNA, 741 bp, synthetic construct
  source 1..741: mol_type = other DNA
ggtgaagatgttgaacaaagcctgagcctgagcgtgcgcgaaggcgatagcgtggttattaattgcacctataccgatagtagcagtacctatctgtattggtataaacaggaaccgggcgcaggtctgcagctgctgacctatattttcagtaatatggatatgaagcaggatcagcgcctgaccgttctgctgaataagaaagataaacatctgagcctgcgtattgccgatgttcagaccggtgacagcgcaatctatttctgtgccgaacagagttttggcaatgaaaagctgacctttggtaccggtacccgtctgaccgttaccccgggtggcggcagtgaaggcggtggtagcgaaggcggcggcagcgaaggtggtggtagtgaaggtggtaccggcaatgccggtgttacccagaccccgaaatatctgagcgttaaaaccggccagagtgttaccctgctgtgcgcccaggatatgaatcatgaatatatgtattggtaccgccaggaccctggccagggtctgcgcttaattcattatagtgtgggtgaaggtaccaccgcaaaaggcgaagtgccggatcgttataatgtgagtcgcctgaagaaacagaattttctgctgggcattgaaagtgtgaccccgagtgataccagcgtgtatttctgtgcaagtagcctgggtcgtgcctatgaacagtattttggcccgggtacccgcctgaccgtgacc

SEQ ID NO: 11 - protein, 205 aa, synthetic construct
GEDVEQSLFLSVREGDSSVINCTYTDSSSTYLYWYKQEPGAGLQLLTYIFSNMDMKQDQRLTVLLNKKDKHLSLRIADTQTGDSAIYFCAEQSFGNEKLTFGTGTRLTIIPNIQNPDPAVYQLRDSKSSDKSVCLFTDFDSQTNVSQSKDSDVYITDKTVLDMRSMDFKSNSAVAWSNKSDFACANAFNNSIIPEDTFFCSPESS

SEQ ID NO: 12 - protein, 242 aa, synthetic construct
NAGVTQTPKFRVLKTGQSMTLLCAQDMNHEYMYWYRQDPGMGLRLIHYSVGEGTTAKGEVPDGYNVSRLKKQNFLLGLESAAPSQTSVYFCASSLGRAYEQYFGPGTRLTVTEDLKNVFPPEVAVFEPSECEISHTQKATLVCLATGFYPDHVELSWWVNGKEVHSGVSTDPQPLKEQPALNDSRYALSSRLRVSATFWQNPRNHFRCQVQFYGLSENDEWTQDRAKPVTQIVSAEAWGRAD

SEQ ID NO: 13 - protein, 111 aa, synthetic construct
GEDVEQSLFLSVREGDSSVINCTYTDSSSTYLYWYKQEPGAGLQLLTYIFSNMDMKQDQRLTVLLNKKDKHLSLRIADTQTGDSAIYFCAEHTKQNEKLTFGTGTRLTIIP

SEQ ID NO: 14 - protein, 111 aa, synthetic construct
GEDVEQSLFLSVREGDSSVINCTYTDSSSTYLYWYKQEPGAGLQLLTYIFSNMDMKQDQRLTVLLNKKDKHLSLRIADTQTGDSAIYFCAWSQFGNEKLTFGTGTRLTIIP

SEQ ID NO: 15 - protein, 111 aa, synthetic construct
GEDVEQSLFLSVREGDSSVINCTYTDSSSTYLYWYKQEPGAGLQLLTYIFSNMDMKQDQRLTVLLNKKDKHLSLRIADTQTGDSAIYFCAVSNFGNEKLTFGTGTRLTIIP

SEQ ID NO: 16 - protein, 111 aa, synthetic construct
GEDVEQSLFLSVREGDSSVINCTYTDSSSTYLYWYKQEPGAGLQLLTYIFSNMDMKQDQRLTVLLNKKDKHLSLRIADTQTGDSAIYFCAASEFGNEKLTFGTGTRLTIIP

SEQ ID NO: 17 - protein, 111 aa, synthetic construct
GEDVEQSLFLSVREGDSSVINCTYTDSSSTYLYWYKQEPGAGLQLLTYIFSNMDMKQDQRLTVLLNKKDKHLSLRIADTQTGDSAIYFCAASTFGNEKLTFGTGTRLTIIP

SEQ ID NO: 18 - protein, 111 aa, synthetic construct
GEDVEQSLFLSVREGDSSVINCTYTDSSSTYLYWYKQEPGAGLQLLTYIFSNMDMKQDQRLTVLLNKKDKHLSLRIADTQTGDSAIYFCAASQFGNEKLTFGTGTRLTIIP

SEQ ID NO: 19 - protein, 111 aa, synthetic construct
GEDVEQSLFLSVREGDSSVINCTYTDSSSTYLYWYKQEPGAGLQLLTYIFSNMDMKQDQRLTVLLNKKDKHLSLRIADTQTGDSAIYFCAASQRGNEKLTFGTGTRLTIIP

SEQ ID NO: 20 - protein, 111 aa, synthetic construct
GEDVEQSLFLSVREGDSSVINCTYTDSSSTYLYWYKQEPGAGLQLLTYIFSNMDMKQDQRLTVLLNKKDKHLSLRIADTQTGDSAIYFCAVSQFGNEKLTFGTGTRLTIIP

SEQ ID NO: 21 - protein, 111 aa, synthetic construct
GEDVEQSLFLSVREGDSSVINCTYTDSSSTYLYWYKQEPGAGLQLLTYIFSNMDMKQDQRLTVLLNKKDKHLSLRIADTQTGDSAIYFCAVSDFGNEKLTFGTGTRLTIIP

SEQ ID NO: 22 - protein, 111 aa, synthetic construct
GEDVEQSLFLSVREGDSSVINCTYTDSSSTYLYWYKQEPGAGLQLLTYIFSNMDMKQDQRLTVLLNKKDKHLSLRIADTQTGDSAIYFCAVSSFGNEKLTFGTGTRLTIIP

SEQ ID NO: 23 - protein, 111 aa, synthetic construct
GEDVEQSLFLSVREGDSSVINCTYTDSSSTYLYWYKQEPGAGLQLLTYIFSNMDMKQDQRLTVLLNKKDKHLSLRIADTQTGDSAIYFCATSTFGNEKLTFGTGTRLTIIP

SEQ ID NO: 24 - protein, 111 aa, synthetic construct
GEDVEQSLFLSVREGDSSVINCTYTDSSSTYLYWYKQEPGAGLQLLTYIFSNMDMKQDQRLTVLLNKKDKHLSLRIADTQTGDSAIYFCATSQFGNEKLTFGTGTRLTIIP

SEQ ID NO: 25 - protein, 111 aa, synthetic construct
GEDVEQSLFLSVREGDSSVINCTYTDSSSTYLYWYKQEPGAGLQLLTYIFSNMDMKQDQRLTVLLNKKDKHLSLRIADTQTGDSAIYFCATSDFGNEKLTFGTGTRLTIIP

SEQ ID NO: 26 - protein, 111 aa, synthetic construct
GEDVEQSLFLSVREGDSSVINCTYTDSSSTYLYWYKQEPGAGLQLLTYIFSNMDMKQDQRLTVLLNKKDKHLSLRIADTQTGDSAIYFCASSQFGNEKLTFGTGTRLTIIP

SEQ ID NO: 27 - protein, 111 aa, synthetic construct
GEDVEQSLFLSVREGDSSVINCTYTDSSSTYLYWYKQEPGAGLQLLTYIFSNMDMKQDQRLTVLLNKKDKHLSLRIADTQTGDSAIYFCAWSSFGNEKLTFGTGTRLTIIP

SEQ ID NO: 28 - protein, 111 aa, synthetic construct
GEDVEQSLFLSVREGDSSVINCTYTDSSSTYLYWYKQEPGAGLQLLTYIFSNMDMKQDQRLTVLLNKKDKHLSLRIADTQTGDSAIYFCAHSQFGNEKLTFGTGTRLTIIP

SEQ ID NO: 29 - protein, 111 aa, synthetic construct
GEDVEQSLFLSVREGDSSVINCTYTDSSSTYLYWYKQEPGAGLQLLTYIFSNMDMKQDQRLTVLLNKKDKHLSLRIADTQTGDSAIYFCAQSQFGNEKLTFGTGTRLTIIP

SEQ ID NO: 30 - protein, 111 aa, synthetic construct
GEDVEQSLFLSVREGDSSVINCTYTDSSSTYLYWYKQEPGAGLQLLTYIFSNMDMKQDQRLTVLLNKKDKHLSLRIADTQTGDSAIYFCANSTFGNEKLTFGTGTRLTIIP

SEQ ID NO: 31 - protein, 111 aa, synthetic construct
GEDVEQSLFLSVREGDSSVINCTYTDSSSTYLYWYKQEPGAGLQLLTYIFSNMDMKQDQRLTVLLNKKDKHLSLRIADTQTGDSAIYFCAYSQFGNEKLTFGTGTRLTIIP

SEQ ID NO: 32 - protein, 111 aa, synthetic construct
GEDVEQSLFLSVREGDSSVINCTYTDSSSTYLYWYKQEPGAGLQLLTYIFSNMDMKQDQRLTVLLNKKDKHLSLRIADTQTGDSAIYFCAEHTHQNEKLTFGTGTRLTIIP

SEQ ID NO: 33 - protein, 205 aa, synthetic construct
GEDVEQSLFLSVREGDSSVINCTYTDSSSTYLYWYKQEPGAGLQLLTYIFSNMDMKQDQRLTVLLNKKDKHLSLRIADTQTGDSAIYFCAEQSFGNEKLTFGTGTRLTIIPNIQNPDPAVYQLRDSKSSDKSVCLFTDFDSQTNVSQSKDSDVYITDKTVLDMRSMDFKSNSAVAWSNKSDFACANAFNNSIIPEDTFFPSPESS

SEQ ID NO: 34 - protein, 242 aa, synthetic construct
NAGVTQTPKFRVLKTGQSMTLLCAQDMNHEYMYWYRQDPGMGLRLIHYSVGEGTTAKGEVPDGYNVSRLKKQNFLLGLESAAPSQTSVYFCASSLGRAYEQYFGPGTRLTVTEDLKNVFPPEVAVFEPSEAEISHTQKATLVCLATGFYPDHVELSWWVNGKEVHSGVSTDPQPLKEQPALNDSRYCLSSRLRVSATFWQNPRNHFRCQVQFYGLSENDEWTQDRAKPVTQIVSAEAWGRAD

SEQ ID NO: 35 - protein, 252 aa, synthetic construct
GEDVEQSLFLSVREGDSSVINCTYTDSSSTYLYWYKQEPGAGLQLLTYIFSNMDMKQDQRLTVLLNKKDKHLSLRIADTQTGDSAIYFCAEQSFGNEKLTFGTGTRLTIIPNIQNPDPAVYQLRDSKSSDKSVCLFTDFDSQTNVSQSKDSDVYITDKTVLDMRSMDFKSNSAVAWSNKSDFACANAFNNSIIPEDTFFPSPESSCDVKLVEKSFETDTNLNFQNLSVIGFRILLLKVAGFNLLMTLRLWSS

SEQ ID NO: 36 - protein, 291 aa, synthetic construct
NAGVTQTPKFRVLKTGQSMTLLCAQDMNHEYMYWYRQDPGMGLRLIHYSVGEGTTAKGEVPDGYNVSRLKKQNFLLGLESAAPSQTSVYFCASSLGRAYEQYFGPGTRLTVTEDLKNVFPPEVAVFEPSEAEISHTQKATLVCLATGFYPDHVELSWWVNGKEVHSGVSTDPQPLKEQPALNDSRYCLSSRLRVSATFWQNPRNHFRCQVQFYGLSENDEWTQDRAKPVTQIVSAEAWGRADCGFTSESYQQGVLSATILYEILLGKATLYAVLVSALVLMAMVKRKDSRG

SEQ ID NO: 37 - protein, 6 aa, synthetic construct
DSSSTY

SEQ ID NO: 38 - protein, 7 aa, synthetic construct
IFSNMDM

SEQ ID NO: 39 - protein, 11 aa, synthetic construct
AEHTKQNEKLT

SEQ ID NO: 40 - protein, 11 aa, synthetic construct
AWSQFGNEKLT

SEQ ID NO: 41 - protein, 11 aa, synthetic construct
AVSNFGNEKLT

SEQ ID NO: 42 - protein, 11 aa, synthetic construct
AASEFGNEKLT

SEQ ID NO: 43 - protein, 11 aa, synthetic construct
AASTFGNEKLT

SEQ ID NO: 44 - protein, 11 aa, synthetic construct
AASQFGNEKLT

SEQ ID NO: 45 - protein, 11 aa, synthetic construct
AASQRGNEKLT

SEQ ID NO: 46 - protein, 11 aa, synthetic construct
AVSQFGNEKLT

SEQ ID NO: 47 - protein, 11 aa, synthetic construct
AVSDFGNEKLT

SEQ ID NO: 48 - protein, 11 aa, synthetic construct
AVSSFGNEKLT

SEQ ID NO: 49 - protein, 11 aa, synthetic construct
ATSTFGNEKLT

SEQ ID NO: 50 - protein, 11 aa, synthetic construct
ATSQFGNEKLT

SEQ ID NO: 51 - protein, 11 aa, synthetic construct
ATSDFGNEKLT

SEQ ID NO: 52 - protein, 11 aa, synthetic construct
ASSQFGNEKLT

SEQ ID NO: 53 - protein, 11 aa, synthetic construct
AWSSFGNEKLT

SEQ ID NO: 54 - protein, 11 aa, synthetic construct
AHSQFGNEKLT

SEQ ID NO: 55 - protein, 11 aa, synthetic construct
AQSQFGNEKLT

SEQ ID NO: 56 - protein, 11 aa, synthetic construct
ANSTFGNEKLT

SEQ ID NO: 57 - protein, 11 aa, synthetic construct
AYSQFGNEKLT

SEQ ID NO: 58 - protein, 11 aa, synthetic construct
AEHTHQNEKLT

SEQ ID NO: 59 - protein, 5 aa, synthetic construct
MNHEY

SEQ ID NO: 60 - protein, 6 aa, synthetic construct
SVGEGT

SEQ ID NO: 61 - protein, 11 aa, synthetic construct
ASSLGRAYEQY

SEQ ID NO: 62 - protein, 11 aa, synthetic construct
AEQSFGNEKLT